European Patent Application EP 4 137 563 A1, published February 22, 2023. Title: NATURAL KILLER CELLS. Applicant: IMPERIAL COLLEGE OF SCIENCE, TECHNOLOGY AND MEDICINE. Application EP. The sequence listing filed with the application follows.

SEQUENCE LISTING (9 sequences)

SEQ ID NO: 1 - DNA, 1923 bp, Homo sapiens
  source 1..1923: mol_type = other DNA
gcccctttctttctcctcgtcggcccgagagcaggaacacgataacgaaggaggcccaacttcattcaataaggagcctgacggatttatcccagacggtagaacaaaaggaagaatattgatggattttaaaccagagtttttaaagagcttgagaatacggggaaattaatttgttctcctacacacatagatagggtaaggttgtttctgatgcagctgagaaaaatgcagaccgtcaaaaaggagcaggcgtctcttgatgccagtagcaatgtggacaagatgatggtccttaattctgctttaacggaagtgtcagaagactccacaacaggtgaggacgtgcttctcagtgaaggaagtgtggggaagaacaaatcttctgcatgtcggaggaaacgggaattcattcctgatgaaaagaaagatgctatgtattgggaaaaaaggcggaaaaataatgaagctgccaaaagatctcgtgagaagcgtcgactgaatgacctggttttagagaacaaactaattgcactgggagaagaaaacgccactttaaaagctgagctgctttcactaaaattaaagtttggtttaattagctccacagcatatgctcaagagattcagaaactcagtaattctacagctgtgtactttcaagattaccagacttccaaatccaatgtgagttcatttgtggacgagcacgaaccctcgatggtgtcaagtagttgtatttctgtcattaaacactctccacaaagctcgctgtccgatgtttcagaagtgtcctcagtagaacacacgcaggagagctctgtgcagggaagctgcagaagtcctgaaaacaagttccagattatcaagcaagagccgatggaattagagagctacacaagggagccaagagatgaccgaggctcttacacagcgtccatctatcaaaactatatggggaattctttctctgggtactcacactctcccccactactgcaagtcaaccgatcctccagcaactccccgagaacgtcggaaactgatgatggtgtggtaggaaagtcatctgatggagaagacgagcaacaggtccccaagggccccatccattctccagttgaactcaagcatgtgcatgcaactgtggttaaagttccagaagtgaattcctctgccttgccacacaagctccggatcaaagccaaagccatgcagatcaaagtagaagcctttgataatgaatttgaggccacgcaaaaactttcctcacctattgacatgacatctaaaagacatttcgaactcgaaaagcatagtgccccaagtatggtacattcttctcttactcctttctcagtgcaagtgactaacattcaagattggtctctcaaatcggagcactggcatcaaaaagaactgagtggcaaaactcagaatagtttcaaaactggagttgttgaaatgaaagacagtggctacaaagtttctgacccagagaacttgtatttgaagcaggggatagcaaacttatctgcagaggttgtctcactcaagagacttatagccacacaaccaatctctgcttcagactctgggtaaattactactgagtaagagctgggcatttagaaagatgtcatttgcaatagagcagtccattttgtattatgctgaattttcactggacctgtgatgtcatttcactgtgatgtgcacatgttgtctgtttggtgtctttttgtgcacagattatgatgaagattagattgtgttatcactctgcctgtgtatagtcagatagtcatatgcgtaaggctgtatatattaagnttttatttttgttgttctattataaagtgtgtaagttaccagtttcaataaaggattggtgacaaacacagaaaaaaaaaaaaaaaaaaa

SEQ ID NO: 2 - protein, 462 aa, Homo sapiens [sequence omitted]

SEQ ID NO: 3 - DNA, 2793 bp, Homo sapiens
  source 1..2793: mol_type = other DNA
gggcacgaggcgctccctgggatcacatggtacctgctccagtgccgcgtgcggcccgggaaccctgggctgctggcgcctgcgcagagccctctgtcccagggaaaggctcgggcaaaaggcggctgagattggcagagtgaaatattactgccgagggaacgtagcagggcacacgtctcgcctctttgcgactcggtgccccgtttctccccatcacctacttacttcctggttgcaacctctcttcctctgggacttttgcaccgggagctccagattcgccaccccgcagcgctgcggagccggcaggcagaggcaccccgtacactgcagagacccgaccctccttgctaccttctagccagaactactgcaggctgattccccctacacactctctctgctcttcccatgcaaagcagaactccgttgcctcaacgtccaacccttctgcagggctgcagtccggccaccccaagaccttgctgcagggtgcttcggatcctgatcgtgagtcgcggggtccactccccgcccttagccagtgcccagggggcaacagcggcgatcgcaacctctagtttgagtcaaggtccagtttgaatgaccgctctcagctggtgaagacatgacgaccctggactccaacaacaacacaggtggcgtcatcacctacattggctccagtggctcctccccaagccgcaccagccctgaatccctctatagtgacaactccaatggcagcttccagtccctgacccaaggctgtcccacctacttcccaccatcccccactggctccctcacccaagacccggctcgctcctttgggagcattccacccagcctgagtgatgacggctccccttcttcctcatcttcctcgtcgtcatcctcctcctccttctataatgggagcccccctgggagtctacaagtggccatggaggacagcagccgagtgtcccccagcaagagcaccagcaacatcaccaagctgaatggcatggtgttactgtgtaaagtgtgtggggacgttgcctcgggcttccactacggtgtgcacgcctgcgagggctgcaagggctttttccgtcggagcatccagcagaacatccagtacaaaaggtgtctgaagaatgagaattgctccatcgtccgcatcaatcgcaaccgctgccagcaatgtcgcttcaagaagtgtctctctgtgggcatgtctcgagacgctgtgcgttttgggcgcatccccaaacgagagaagcagcggatgcttgctgagatgcagagtgccatgaacctggccaacaaccagttgagcagccagtgcccgctggagacttcacccacccagcaccccaccccaggccccatgggcccctcgccaccccctgctccggtcccctcacccctggtgggcttctcccagtttccacaacagctgacgcctcccagatccccaagccctgagcccacagtggaggatgtgatatcccaggtggcccgggcccatcgagagatcttcacctacgcccatgacaagctgggcagctcacctggcaacttcaatgccaaccatgcatcaggtagccctccagccaccaccccacatcgctgggaaaatcagggctgcccacctgcccccaatgacaacaacaccttggctgcccagcgtcataacgaggccctaaatggtctgcgccaggctccctcctcctaccctcccacctggcctcctggccctgcacaccacagctgccaccagtccaacagcaacgggcaccgtctatgccccacccacgtgtatgcagccccagaaggcaaggcacctgccaacagtccccggcagggcaactcaaagaatgttctgctggcatgtcctatgaacatgtacccgcatggacgcagtgggcgaacggtgcaggagatctgggaggatttctccatgagcttcacgcccgctgtgcgggaggtggtagagtttgccaaacacatcccgggcttccgtgacctttctcagcatgaccaagtcaccctgcttaaggctggcacctttgaggtgctgatggtgcgctttgcttcgttgttcaacgtgaaggaccagacagtgatgttcctaagccgcaccacctacagcctgcaggagcttggtgccatgggcatgggagacctgctcagtgccatgttcgacttcagcgagaagctcaactccctggcgcttaccgaggaggagctgggcctcttcaccgcggtggtgcttgtctctgcagaccgctcgggcatggagaattccgcttcggtggagcagctccaggagacgctgctgcgggctcttcgggctctggtgctgaagaaccggcccttggagacttcccgcttcaccaagctgctgctcaagctgccggacctgcggaccctgaacaacatgcattccgagaagctgctgtccttccgggtggacgcccagtgacccgcccggccggccttctgccgctgcccccttgtacagaatcgaactctgcacttctctctcctttacgagacgaaaaggaaaagcaaaccagaatcttatttatattgttataaaatattccaagatgagcctctggccccctgagccttcttgtaaatacctgcctccctcccccatcaccgaacttcccctcctcccctatttaaaccactctgtctcccccacaaccctcccctggccctctgatttgttctgttcctgtctcaaatccaatagttcacagctgagctggcttcaaaaaaaaaaaaaaaaaa

SEQ ID NO: 4 - protein, 614 aa, Homo sapiens
MTTLDSNNNTGGVITYIGSSGSSPSRTSPESLYSDNSNGSFQSLTQGCPTYFPPSPTGSLTQDPARSFGSIPPSLSDDGSPSSSSSSSSSSSSFYNGSPPGSLQVAMEDSSRVSPSKSTSNITKLNGMVLLCKVCGDVASGFHYGVHACEGCKGFFRRSIQQNIQYKRCLKNENCSIVRINRNRCQQCRFKKCLSVGMSRDAVRFGRIPKREKQRMLAEMQSAMNLANNQLSSQCPLETSPTQHPTPGPMGPSPPPAPVPSPLVGFSQFPQQLTPPRSPSPEPTVEDVISQVARAHREIFTYAHDKLGSSPGNFNANHASGSPPATTPHRWENQGCPPAPNDNNTLAAQRHNEALNGLRQAPSSYPPTWPPGPAHHSCHQSNSNGHRLCPTHVYAAPEGKAPANSPRQGNSKNVLLACPMNMYPHGRSGRTVQEIWEDFSMSFTPAVREVVEFAKHIPGFRDLSQHDQVTLLKAGTFEVLMVRFASLFNVKDQTVMFLSRTTYSLQELGAMGMGDLLSAMFDFSEKLNSLALTEEELGLFTAVVLVSADRSGMENSASVEQLQETLLRALRALVLKNRPLETSRFTKLLLKLPDLRTLNNMHSEKLLSFRVDAQ

SEQ ID NO: 5 - DNA, 1740 bp, Homo sapiens
  source 1..1740: mol_type = other DNA
atggaggtgaatgcaggaggtgtgattgcctatatcagttcttccagctcagcctcaagccctgcctcttgtcacagtgagggttctgagaatagtttccagtcctcctcctcttctgttccatcttctccaaatagctctaattctgataccaatggtaatcccaagaatggtgatctcgccaatattgaaggcatcttgaagaatgatcgaatagattgttctatgaaaacaagcaaatcgagtgcacctgggatgacaaaaaatcatagtggtgtgacaaaatttagtggcatggttctactgtgtaaagtctgtggggatgtggcgtcaggattccactatggagttcatgcttgcgaaggctgtaagggtttctttcggagaagtattcaacaaaacatccagtacaagaagtgcctgaagaatgaaaactgttctataatgagaatgaataggaacagatgtcagcaatgtcgcttcaaaaagtgtctgtctgttggaatgtcaagagatgctgttcggtttggtcgtattcctaagcgtgaaaaacagaggatgctaattgaaatgcaaagtgcaatgaagaccatgatgaacagccagttcagtggtcacttgcaaaatgacacattagtagaacatcatgaacagacagccttgccagcccaggaacagctgcgacccaagccccaactggagcaagaaaacatcaaaagctcttctcctccatcttctgattttgcaaaggaagaagtgattggcatggtgaccagagctcacaaggatacctttatgtataatcaagagcagcaagaaaactcagctgagagcatgcagccccagagaggagaacggattcccaagaacatggagcaatataatttaaatcatgatcattgcggcaatgggcttagcagccattttccctgtagtgagagccagcagcatctcaatggacagttcaaagggaggaatataatgcattacccanatggccatgccatttgtattgcaaatggacattgtatgaacttctccaatgcttatactcaaagagtatgtgatagagttccgatagatggattttctcagaatgagaacaagaatagttacctgtgcaacactggaggaagaatgcatctggtttgtccaatgagtaagtctccatatgtggatcctcataaatcaggacatgaaatctgggaagaattttcgatgagcttcactccagcagtgaaagaagtggtggaatttgcaaagcgtattcctgggttcagagatctctctcagcatgaccaggtcaaccttttaaaggctgggacttttgaggttttaatggtacggttcgcatcattatttgatgcaaaggaacgtactgtcacctttttaagtggaaagaaatatagtgtggatgatttacactcaatgggagcaggggatctgctaaactctatgtttgaatttagtgagaagctaaatgccctccaacttagtgatgaagagatgagtttgtttacagctgttgtcctggtatctgcagatcgatctggaatagaaaacgtcaactctgtggaggctttgcaggaaactctcattcgtgcactaaggaccttaataatgaaaaaccatccaaatgaggcctctatttttacaaaactgcttctaaagttgccagatcttcgatctttaaacaacatgcactctgaggagctcttggcctttaaagttcacccttaa

SEQ ID NO: 6 - protein, 578 aa, Homo sapiens
MEVNAGGVIAYISSSSSASSPASCHSEGSENSFQSSSSSVPSSPNSSNSDTNGNPKNGDLANIEGILKNDRIDCSMKTSKSSAPGMTKNHSGVTKFSGMVLLCKVCGDVASGFHYGVHACEGCKGFFRRSIQQNIQYKKCLKNENCSIMRMNRNRCQQCRFKKCLSVGMSRDAVRFGRIPKREKQRMLIEMQSAMKTMMNSQFSGHLQNDTLVEHHEQTALPAQEQLRPKPQLEQENIKSSSPPSSDFAKEEVIGMVTRAHKDTFMYNQEQQENSAESMQPQRGERIPKNMEQYNLNHDHCGNGLSSHFPCSESQQHLNGQFKGRNIMHYPXGHAICIANGHCMNFSNAYTQRVCDRVPIDGFSQNENKNSYLCNTGGRMHLVCPMSKSPYVDPHKSGHEIWEEFSMSFTPAVKEVVEFAKRIPGFRDLSQHDQVNLLKAGTFEVLMVRFASLFDAKERTVTFLSGKKYSVDDLHSMGAGDLLNSMFEFSEKLNALQLSDEEMSLFTAVVLVSADRSGIENVNSVEALQETLIRALRTLIMKNHPNEASIFTKLLLKLPDLRSLNNMHSEELLAFKVH

SEQ ID NO: 7 - DNA, 20 bp, synthetic construct
  misc_feature 1..20: note = forward primer A for detection of E4bp4 wildtype allele
  source 1..20: mol_type = other DNA
ctctgagcttggctgatgtg

SEQ ID NO: 8 - DNA, 20 bp, synthetic construct
  misc_feature 1..20: note = reverse primer for the detection of E4bp4
  source 1..20: mol_type = other DNA
gcttcaagtctccaccaagc

SEQ ID NO: 9 - DNA, 20 bp, synthetic construct
  misc_feature 1..20: note = primer for the detection of the E4bp4 null allele
  source 1..20: mol_type = other DNA
ccatgctcctgtcttgatga